European Patent Application EP 4 218 928 A2, published August 2, 2023. Title: SELF-ASSEMBLING PEPTIDE SCAFFOLD. Applicant: Amplicon Vaccine, LLC. The sequence listing filed with the application follows.

SEQUENCE LISTING (20 sequences)

SEQ ID NO: 1 - protein, 7 aa, synthetic construct
  REGION 1..7: note = heptad
LRSIGKD

SEQ ID NO: 2 - protein, 7 aa, synthetic construct
  REGION 1..7: note = heptad
LRSIGRD

SEQ ID NO: 3 - protein, 7 aa, synthetic construct
  REGION 1..7: note = heptad
IREISRA

SEQ ID NO: 4 - protein, 7 aa, synthetic construct
  REGION 1..7: note = heptad
IREVAQS

SEQ ID NO: 5 - protein, 7 aa, synthetic construct
  REGION 1..7: note = heptad
IRDIAKA

SEQ ID NO: 6 - protein, 7 aa, synthetic construct
  REGION 1..7: note = heptad
IRDIGRA

SEQ ID NO: 7 - protein, 7 aa, synthetic construct
  REGION 1..7: note = heptad
IRDVGQS

SEQ ID NO: 8 - protein, 7 aa, synthetic construct
  REGION 1..7: note = heptad
IRDLAKG

SEQ ID NO: 9 - protein, 7 aa, synthetic construct
  REGION 1..7: note = heptad
VKDVARG

SEQ ID NO: 10 - protein, 7 aa, synthetic construct
  REGION 1..7: note = heptad
IRDIGNS

SEQ ID NO: 11 - protein, 7 aa, synthetic construct
  REGION 1..7: note = heptad
IKDLARG

SEQ ID NO: 12 - protein, 7 aa, synthetic construct
  REGION 1..7: note = heptad
IKKLKKK

SEQ ID NO: 13 - protein, 28 aa, synthetic construct
  REGION 1..28: note = hexamer
LRSIGKDLRSIGKDLRSIGKDLRSIGKD

SEQ ID NO: 14 - protein, 29 aa, synthetic construct
  REGION 1..29: note = hexamer
LRSIGKDLRSIGKDLRSIGKDLRSIGKDS

SEQ ID NO: 15 - protein, 28 aa, synthetic construct
  REGION 1..28: note = hexamer
LRSIGKDLRSIGRDLRSIGKDLRSIGRD

SEQ ID NO: 16 - protein, 28 aa, synthetic construct
  REGION 1..28: note = hexamer
IREISRAIREVAQSIRDIAKAIREIGKS

SEQ ID NO: 17 - protein, 28 aa, synthetic construct
  REGION 1..28: note = hexamer
IRDIGRAIRDVGQSIRDLAKGIRDISKG

SEQ ID NO: 18 - protein, 28 aa, synthetic construct
  REGION 1..28: note = hexamer
VKDVARGIRDIGNSIKDLARGIRDIGRG

SEQ ID NO: 19-20 - skipped (2 entries)